European Patent Specification EP 3 985 019 B1, published September 18, 2024. Title: Recombinant Human Collagen and Construction Method Therefor. Applicant: Nantong University. Application EP20932054.8. The sequence listing filed with the application follows.

SEQUENCE LISTING (1 sequence)

SEQ ID NO: 1 - protein, 30 aa, Artificial Sequence
  rh collagen
GPAGARGNDGATGAAGPPGPTGPAGPPGFP